European Patent Application EP 4 275 747 A2, published November 15, 2023. Title: THERAPEUTIC APPLICATIONS OF CPF1-BASED GENOME EDITING. Applicant: DUKE UNIVERSITY. The sequence listing filed with the application follows.

SEQUENCE LISTING (125 sequences)

SEQ ID NO: 1 - DNA, 27 bp, Homo sapiens
  source 1..27: mol_type = other DNA
tttgcaaaaacccaaaatattttagct

SEQ ID NO: 2 - DNA, 27 bp, Homo sapiens
  source 1..27: mol_type = other DNA
tttgcctttttggtatcttacaggaac

SEQ ID NO: 3 - DNA, 27 bp, Homo sapiens
  source 1..27: mol_type = other DNA
tccaggatggcattgggcagcggcaaa

SEQ ID NO: 4 - DNA, 27 bp, Homo sapiens
  source 1..27: mol_type = other DNA
tttatttttccttttattctagttgaa

SEQ ID NO: 5 - DNA, 27 bp, Homo sapiens
  source 1..27: mol_type = other DNA
tttcttgatccatatgcttttacctgc

SEQ ID NO: 6 - DNA, 27 bp, Homo sapiens
  source 1..27: mol_type = other DNA
aggcgatttgacagatctgttgagaaa

SEQ ID NO: 7 - DNA, 27 bp, Homo sapiens
  source 1..27: mol_type = other DNA
tttattcttctttctccaggctagaag

SEQ ID NO: 8 - DNA, 27 bp, Homo sapiens
  source 1..27: mol_type = other DNA
ttctttctccaggctagaagaacaaaa

SEQ ID NO: 9 - DNA, 27 bp, Homo sapiens
  source 1..27: mol_type = other DNA
tacaggcaacaatgcaggatttggaac

SEQ ID NO: 10 - DNA, 27 bp, Homo sapiens
  source 1..27: mol_type = other DNA
ttttctgttaaagaggaagttagaaga

SEQ ID NO: 11 - DNA, 27 bp, Homo sapiens
  source 1..27: mol_type = other DNA
ttttaaaatttttatattacagaatat

SEQ ID NO: 12 - DNA, 27 bp, Homo sapiens
  source 1..27: mol_type = other DNA
agaatataaaagatagtctacaacaaa

SEQ ID NO: 13 - DNA, 27 bp, Homo sapiens
  source 1..27: mol_type = other DNA
tttattttgcattttagatgaaagaga

SEQ ID NO: 14 - DNA, 27 bp, Homo sapiens
  source 1..27: mol_type = other DNA
ttttagatgaaagagaagatgttcaaa

SEQ ID NO: 15 - DNA, 27 bp, Homo sapiens
  source 1..27: mol_type = other DNA
gatgaaagagaagatgttcaaaagaaa

SEQ ID NO: 16 - DNA, 27 bp, Homo sapiens
  source 1..27: mol_type = other DNA
tttgcaaaaacccaaaatattttagct

SEQ ID NO: 17 - DNA, 27 bp, Homo sapiens
  source 1..27: mol_type = other DNA
tttagcttgtgtttctaatttttcttt

SEQ ID NO: 18 - DNA, 27 bp, Homo sapiens
  source 1..27: mol_type = other DNA
tttgacttattgttattgaaattggct

SEQ ID NO: 19 - DNA, 27 bp, Homo sapiens
  source 1..27: mol_type = other DNA
tttctaccatgtattgctaaacaaagt

SEQ ID NO: 20 - DNA, 27 bp, Homo sapiens
  source 1..27: mol_type = other DNA
tttagtatcaattcacaccagcaagtt

SEQ ID NO: 21 - DNA, 27 bp, Homo sapiens
  source 1..27: mol_type = other DNA
ataatcgccactttacagaggagtaaa

SEQ ID NO: 22 - DNA, 27 bp, Homo sapiens
  source 1..27: mol_type = other DNA
tttctttaaaatgaagattttccacca

SEQ ID NO: 23 - DNA, 27 bp, Homo sapiens
  source 1..27: mol_type = other DNA
tttaaaatgaagattttccaccaatca

SEQ ID NO: 24 - DNA, 27 bp, Homo sapiens
  source 1..27: mol_type = other DNA
ttttccaccaatcactttactctccta

SEQ ID NO: 25 - DNA, 27 bp, Homo sapiens
  source 1..27: mol_type = other DNA
tttcccaccagttcttaggcaactgtt

SEQ ID NO: 26 - DNA, 27 bp, Homo sapiens
  source 1..27: mol_type = other DNA
ataatcaaggatataaattaatgcaaa

SEQ ID NO: 27 - DNA, 27 bp, Homo sapiens
  source 1..27: mol_type = other DNA
ttttgttgttgttgttaaggtcaaagt

SEQ ID NO: 28 - DNA, 27 bp, Homo sapiens
  source 1..27: mol_type = other DNA
tttaaaattaccctagatcttaaagtt

SEQ ID NO: 29 - DNA, 28 bp, Homo sapiens
  source 1..28: mol_type = other DNA
cacgcccccaccctaatcagaggccaaa

SEQ ID NO: 30 - DNA, 28 bp, Homo sapiens
  source 1..28: mol_type = other DNA
ccaaacccttcctggagcctgtgataaa

SEQ ID NO: 31 - DNA, 28 bp, Homo sapiens
  source 1..28: mol_type = other DNA
ccttccgaaagaggcccccctgggcaaa

SEQ ID NO: 32 - DNA, 28 bp, Homo sapiens
  source 1..28: mol_type = other DNA
tctccatcaccaagagagccttccgaaa

SEQ ID NO: 33 - DNA, 28 bp, Homo sapiens
  source 1..28: mol_type = other DNA
tgttagcttgcactagactagcttcaaa

SEQ ID NO: 34 - DNA, 28 bp, Homo sapiens
  source 1..28: mol_type = other DNA
ttttctggcctatgttattacctgtatg

SEQ ID NO: 35 - DNA, 28 bp, Homo sapiens
  source 1..28: mol_type = other DNA
tttctggcctatgttattacctgtatgg

SEQ ID NO: 36 - DNA, 23 bp, synthetic construct
  source 1..23: mol_type = other DNA
caaaaacccaaaatattttagct

SEQ ID NO: 37 - DNA, 23 bp, synthetic construct
  source 1..23: mol_type = other DNA
cctttttggtatcttacaggaac

SEQ ID NO: 38 - DNA, 23 bp, synthetic construct
  source 1..23: mol_type = other DNA
ccgctgcccaatgccatcctgga

SEQ ID NO: 39 - DNA, 23 bp, synthetic construct
  source 1..23: mol_type = other DNA
tttttccttttattctagttgaa

SEQ ID NO: 40 - DNA, 23 bp, synthetic construct
  source 1..23: mol_type = other DNA
ttgatccatatgcttttacctgc

SEQ ID NO: 41 - DNA, 23 bp, synthetic construct
  source 1..23: mol_type = other DNA
tcaacagatctgtcaaatcgcct

SEQ ID NO: 42 - DNA, 23 bp, synthetic construct
  source 1..23: mol_type = other DNA
ttcttctttctccaggctagaag

SEQ ID NO: 43 - DNA, 23 bp, synthetic construct
  source 1..23: mol_type = other DNA
gttcttctagcctggagaaagaa

SEQ ID NO: 44 - DNA, 23 bp, synthetic construct
  source 1..23: mol_type = other DNA
caaatcctgcattgttgcctgta

SEQ ID NO: 45 - DNA, 23 bp, synthetic construct
  source 1..23: mol_type = other DNA
ctgttaaagaggaagttagaaga

SEQ ID NO: 46 - DNA, 23 bp, synthetic construct
  source 1..23: mol_type = other DNA
aaaatttttatattacagaatat

SEQ ID NO: 47 - DNA, 23 bp, synthetic construct
  source 1..23: mol_type = other DNA
ttgtagactatcttttatattct

SEQ ID NO: 48 - DNA, 23 bp, synthetic construct
  source 1..23: mol_type = other DNA
ttttgcattttagatgaaagaga

SEQ ID NO: 49 - DNA, 23 bp, synthetic construct
  source 1..23: mol_type = other DNA
aacatcttctctttcatctaaaa

SEQ ID NO: 50 - DNA, 23 bp, synthetic construct
  source 1..23: mol_type = other DNA
ttttgaacatcttctctttcatc

SEQ ID NO: 51 - DNA, 23 bp, synthetic construct
  source 1..23: mol_type = other DNA
caaaaacccaaaatattttagct

SEQ ID NO: 52 - DNA, 23 bp, synthetic construct
  source 1..23: mol_type = other DNA
gcttgtgtttctaatttttcttt

SEQ ID NO: 53 - DNA, 23 bp, synthetic construct
  source 1..23: mol_type = other DNA
acttattgttattgaaattggct

SEQ ID NO: 54 - DNA, 23 bp, synthetic construct
  source 1..23: mol_type = other DNA
taccatgtattgctaaacaaagt

SEQ ID NO: 55 - DNA, 23 bp, synthetic construct
  source 1..23: mol_type = other DNA
gtatcaattcacaccagcaagtt

SEQ ID NO: 56 - DNA, 23 bp, synthetic construct
  source 1..23: mol_type = other DNA
ctcctctgtaaagtggcgattat

SEQ ID NO: 57 - DNA, 23 bp, synthetic construct
  source 1..23: mol_type = other DNA
tttaaaatgaagattttccacca

SEQ ID NO: 58 - DNA, 23 bp, synthetic construct
  source 1..23: mol_type = other DNA
aaatgaagattttccaccaatca

SEQ ID NO: 59 - DNA, 23 bp, synthetic construct
  source 1..23: mol_type = other DNA
ccaccaatcactttactctccta

SEQ ID NO: 60 - DNA, 23 bp, synthetic construct
  source 1..23: mol_type = other DNA
ccaccagttcttaggcaactgtt

SEQ ID NO: 61 - DNA, 23 bp, synthetic construct
  source 1..23: mol_type = other DNA
cattaatttatatccttgattat

SEQ ID NO: 62 - DNA, 23 bp, synthetic construct
  source 1..23: mol_type = other DNA
gttgttgttgttaaggtcaaagt

SEQ ID NO: 63 - DNA, 23 bp, synthetic construct
  source 1..23: mol_type = other DNA
aaattaccctagatcttaaagtt

SEQ ID NO: 64 - DNA, 24 bp, synthetic construct
  source 1..24: mol_type = other DNA
gcctctgattagggtgggggcgtg

SEQ ID NO: 65 - DNA, 24 bp, synthetic construct
  source 1..24: mol_type = other DNA
tcacaggctccaggaagggtttgg

SEQ ID NO: 66 - DNA, 24 bp, synthetic construct
  source 1..24: mol_type = other DNA
cccaggggggcctctttcggaagg

SEQ ID NO: 67 - DNA, 24 bp, synthetic construct
  source 1..24: mol_type = other DNA
ggaaggctctcttggtgatggaga

SEQ ID NO: 68 - DNA, 24 bp, synthetic construct
  source 1..24: mol_type = other DNA
aagctagtctagtgcaagctaaca

SEQ ID NO: 69 - DNA, 24 bp, synthetic construct
  source 1..24: mol_type = other DNA
ctggcctatgttattacctgtatg

SEQ ID NO: 70 - DNA, 24 bp, synthetic construct
  source 1..24: mol_type = other DNA
tggcctatgttattacctgtatgg

SEQ ID NO: 71 - DNA, 23 bp, synthetic construct
  source 1..23: mol_type = other DNA
ttccattctaatgggtggctgtt

SEQ ID NO: 72 - DNA, 20 bp, synthetic construct
  source 1..20: mol_type = other DNA
ctcctctgtaaagtggcgat

SEQ ID NO: 73 - DNA, 20 bp, synthetic construct
  source 1..20: mol_type = other DNA
ttccattctaatgggtggct

SEQ ID NO: 74 - DNA, 20 bp, synthetic construct
  source 1..20: mol_type = other DNA
gtatcaattcacaccagcaa

SEQ ID NO: 75 - DNA, 20 bp, synthetic construct
  source 1..20: mol_type = other DNA
taccatgtattgctaaacaa

SEQ ID NO: 76 - DNA, 20 bp, synthetic construct
  source 1..20: mol_type = other DNA
acttattgttattgaaattg

SEQ ID NO: 77 - DNA, 20 bp, synthetic construct
  source 1..20: mol_type = other DNA
gcttgtgtttctaatttttc

SEQ ID NO: 78 - DNA, 20 bp, synthetic construct
  source 1..20: mol_type = other DNA
caaaaacccaaaatatttta

SEQ ID NO: 79 - DNA, 20 bp, synthetic construct
  source 1..20: mol_type = other DNA
tttaaaatgaagattttcca

SEQ ID NO: 80 - DNA, 20 bp, synthetic construct
  source 1..20: mol_type = other DNA
aaatgaagattttccaccaa

SEQ ID NO: 81 - DNA, 20 bp, synthetic construct
  source 1..20: mol_type = other DNA
ccaccaatcactttactctc

SEQ ID NO: 82 - DNA, 20 bp, synthetic construct
  source 1..20: mol_type = other DNA
ccaccagttcttaggcaact

SEQ ID NO: 83 - DNA, 20 bp, synthetic construct
  source 1..20: mol_type = other DNA
cattaatttatatccttgat

SEQ ID NO: 84 - DNA, 20 bp, synthetic construct
  source 1..20: mol_type = other DNA
agttatagctctctttcaat

SEQ ID NO: 85 - DNA, 20 bp, synthetic construct
  source 1..20: mol_type = other DNA
atgtataacaattccaacat

SEQ ID NO: 86 - DNA, 20 bp, synthetic construct
  source 1..20: mol_type = other DNA
aaattaccctagatcttaaa

SEQ ID NO: 87 - DNA, 20 bp, synthetic construct
  source 1..20: mol_type = other DNA
gttgttgttgttaaggtcaa

SEQ ID NO: 88 - DNA, 20 bp, synthetic construct
  source 1..20: mol_type = other DNA
gcttgtgtttctaatttttc

SEQ ID NO: 89 - DNA, 20 bp, synthetic construct
  source 1..20: mol_type = other DNA
taatttttctttttcttctt

SEQ ID NO: 90 - DNA, 20 bp, synthetic construct
  source 1..20: mol_type = other DNA
gcaaaaaggaaaaaagaaga

SEQ ID NO: 91 - DNA, 20 bp, synthetic construct
  source 1..20: mol_type = other DNA
gggtttttgcaaaaaggaaa

SEQ ID NO: 92 - DNA, 20 bp, synthetic construct
  source 1..20: mol_type = other DNA
agctcctactcagactgtta

SEQ ID NO: 93 - DNA, 20 bp, synthetic construct
  source 1..20: mol_type = other DNA
tgcaaaaacccaaaatattt

SEQ ID NO: 94 - DNA, 20 bp, synthetic construct
  source 1..20: mol_type = other DNA
tgtcaccagagtaacagtct

SEQ ID NO: 95 - DNA, 20 bp, synthetic construct
  source 1..20: mol_type = other DNA
cttagtaaccacaggttgtg

SEQ ID NO: 96 - DNA, 20 bp, synthetic construct
  source 1..20: mol_type = other DNA
tagtttggagatggcagttt

SEQ ID NO: 97 - DNA, 20 bp, synthetic construct
  source 1..20: mol_type = other DNA
gagatggcagtttccttagt

SEQ ID NO: 98 - DNA, 20 bp, synthetic construct
  source 1..20: mol_type = other DNA
cttgatgttggaggtacctg

SEQ ID NO: 99 - DNA, 20 bp, synthetic construct
  source 1..20: mol_type = other DNA
atgttggaggtacctgctct

SEQ ID NO: 100 - DNA, 20 bp, synthetic construct
  source 1..20: mol_type = other DNA
taacttgatcaagcagagaa

SEQ ID NO: 101 - DNA, 20 bp, synthetic construct
  source 1..20: mol_type = other DNA
tctgcttgatcaagttataa

SEQ ID NO: 102 - DNA, 20 bp, synthetic construct
  source 1..20: mol_type = other DNA
taaaatcacagagggtgatg

SEQ ID NO: 103 - DNA, 20 bp, synthetic construct
  source 1..20: mol_type = other DNA
atatcctcaaggtcacccac

SEQ ID NO: 104 - DNA, 20 bp, synthetic construct
  source 1..20: mol_type = other DNA
atgatcatctcgttgatatc

SEQ ID NO: 105 - DNA, 20 bp, synthetic construct
  source 1..20: mol_type = other DNA
tcataccttctgcttgatga

SEQ ID NO: 106 - DNA, 20 bp, synthetic construct
  source 1..20: mol_type = other DNA
tcattttttctcataccttc

SEQ ID NO: 107 - DNA, 20 bp, synthetic construct
  source 1..20: mol_type = other DNA
tgccaacttttatcattttt

SEQ ID NO: 108 - DNA, 20 bp, synthetic construct
  source 1..20: mol_type = other DNA
aatcagaaagaagatcttat

SEQ ID NO: 109 - DNA, 20 bp, synthetic construct
  source 1..20: mol_type = other DNA
atttccctagggtccagctt

SEQ ID NO: 110 - DNA, 20 bp, synthetic construct
  source 1..20: mol_type = other DNA
gctcaaattgttactcttca

SEQ ID NO: 111 - DNA, 20 bp, synthetic construct
  source 1..20: mol_type = other DNA
agctcctactcagactgtta

SEQ ID NO: 112 - DNA, 20 bp, synthetic construct
  source 1..20: mol_type = other DNA
attctagtactatgcatctt

SEQ ID NO: 113 - DNA, 20 bp, synthetic construct
  source 1..20: mol_type = other DNA
acttaagttacttgtccagg

SEQ ID NO: 114 - DNA, 20 bp, synthetic construct
  source 1..20: mol_type = other DNA
ccaaggtcccagagttccta

SEQ ID NO: 115 - DNA, 20 bp, synthetic construct
  source 1..20: mol_type = other DNA
tttccctggcaaggtctgaa

SEQ ID NO: 116 - DNA, 20 bp, synthetic construct
  source 1..20: mol_type = other DNA
gctcattctcatgcctggac

SEQ ID NO: 117 - DNA, 20 bp, synthetic construct
  source 1..20: mol_type = other DNA
tttagcaatacatggtagaa

SEQ ID NO: 118 - DNA, 20 bp, synthetic construct
  source 1..20: mol_type = other DNA
agccaaactcttattcatga

SEQ ID NO: 119 - DNA, 20 bp, synthetic construct
  source 1..20: mol_type = other DNA
taacaatgtggatactttgt

SEQ ID NO: 120-123 - skipped (4 entries)

SEQ ID NO: 124 - DNA, 9464 bp, synthetic construct
  source 1..9464: mol_type = other DNA
gacggatcgggagatctcccgatcccctatggtgcactctcagtacaatctgctctgatgccgcatagttaagccagtatctgctccctgcttgtgtgttggaggtcgctgagtagtgcgcgagcaaaatttaagctacaacaaggcaaggcttgaccgacaattgcatgaagaatctgcttagggttaggcgttttgcgctgcttcgcgatgtacgggccagatatacgcgttgacattgattattgactagttattaatagtaatcaattacggggtcattagttcatagcccatatatggagttccgcgttacataacttacggtaaatggcccgcctggctgaccgcccaacgacccccgcccattgacgtcaataatgacgtatgttcccatagtaacgccaatagggactttccattgacgtcaatgggtggagtatttacggtaaactgcccacttggcagtacatcaagtgtatcatatgccaagtacgccccctattgacgtcaatgacggtaaatggcccgcctggcattatgcccagtacatgaccttatgggactttcctacttggcagtacatctacgtattagtcatcgctattaccatggtgatgcggttttggcagtacatcaatgggcgtggatagcggtttgactcacggggatttccaagtctccaccccattgacgtcaatgggagtttgttttggcaccaaaatcaacgggactttccaaaatgtcgtaacaactccgccccattgacgcaaatgggcggtaggcgtgtacggtgggaggtctatataagcagagctctctggctaactagagaacccactgcttactggcttatcgaaattaatacgactcactatagggagacccaagctggctagcgtttaaacttaagcttggtaccgccaccatgacacagttcgagggctttaccaacctgtatcaggtgagcaagacactgcggtttgagctgatcccacagggcaagaccctgaagcacatccaggagcagggcttcatcgaggaggacaaggcccgcaatgatcactacaaggagctgaagcccatcatcgatcggatctacaagacctatgccgaccagtgcctgcagctggtgcagctggattgggagaacctgagcgccgccatcgactcctatagaaaggagaaaaccgaggagacaaggaacgccctgatcgaggagcaggccacatatcgcaatgccatccacgactacttcatcggccggacagacaacctgaccgatgccatcaataagagacacgccgagatctacaagggcctgttcaaggccgagctgtttaatggcaaggtgctgaagcagctgggcaccgtgaccacaaccgagcacgagaacgccctgctgcggagcttcgacaagtttacaacctacttctccggcttttatgagaacaggaagaacgtgttcagcgccgaggatatcagcacagccatcccacaccgcatcgtgcaggacaacttccccaagtttaaggagaattgtcacatcttcacacgcctgatcaccgccgtgcccagcctgcgggagcactttgagaacgtgaagaaggccatcggcatcttcgtgagcacctccatcgaggaggtgttttccttccctttttataaccagctgctgacacagacccagatcgacctgtataaccagctgctgggaggaatctctcgggaggcaggcaccgagaagatcaagggcctgaacgaggtgctgaatctggccatccagaagaatgatgagacagcccacatcatcgcctccctgccacacagattcatccccctgtttaagcagatcctgtccgataggaacaccctgtctttcatcctggaggagtttaagagcgacgaggaagtgatccagtccttctgcaagtacaagacactgctgagaaacgagaacgtgctggagacagccgaggccctgtttaacgagctgaacagcatcgacctgacacacatcttcatcagccacaagaagctggagacaatcagcagcgccctgtgcgaccactgggatacactgaggaatgccctgtatgagcggagaatctccgagctgacaggcaagatcaccaagtctgccaaggagaaggtgcagcgcagcctgaagcacgaggatatcaacctgcaggagatcatctctgccgcaggcaaggagctgagcgaggccttcaagcagaaaaccagcgagatcctgtcccacgcacacgccgccctggatcagccactgcctacaaccctgaagaagcaggaggagaaggagatcctgaagtctcagctggacagcctgctgggcctgtaccacctgctggactggtttgccgtggatgagtccaacgaggtggaccccgagttctctgcccggctgaccggcatcaagctggagatggagccttctctgagcttctacaacaaggccagaaattatgccaccaagaagccctactccgtggagaagttcaagctgaactttcagatgcctacactggcctctggctgggacgtgaataaggagaagaacaatggcgccatcctgtttgtgaagaacggcctgtactatctgggcatcatgccaaagcagaagggcaggtataaggccctgagcttcgagcccacagagaaaaccagcgagggctttgataagatgtactatgactacttccctgatgccgccaagatgatcccaaagtgcagcacccagctgaaggccgtgacagcccactttcagacccacacaacccccatcctgctgtccaacaatttcatcgagcctctggagatcacaaaggagatctacgacctgaacaatcctgagaaggagccaaagaagtttcagacagcctacgccaagaaaaccggcgaccagaagggctacagagaggccctgtgcaagtggatcgacttcacaagggattttctgtccaagtataccaagacaacctctatcgatctgtctagcctgcggccatcctctcagtataaggacctgggcgagtactatgccgagctgaatcccctgctgtaccacatcagcttccagagaatcgccgagaaggagatcatggatgccgtggagacaggcaagctgtacctgttccagatctataacaaggactttgccaagggccaccacggcaagcctaatctgcacacactgtattggaccggcctgttttctccagagaacctggccaagacaagcatcaagctgaatggccaggccgagctgttctaccgccctaagtccaggatgaagaggatggcacaccggctgggagagaagatgctgaacaagaagctgaaggatcagaaaaccccaatccccgacaccctgtaccaggagctgtacgactatgtgaatcacagactgtcccacgacctgtctgatgaggccagggccctgctgcccaacgtgatcaccaaggaggtgtctcacgagatcatcaaggataggcgctttaccagcgacaagttctttttccacgtgcctatcacactgaactatcaggccgccaattccccatctaagttcaaccagagggtgaatgcctacctgaaggagcaccccgagacacctatcatcggcatcgatcggggcgagagaaacctgatctatatcacagtgatcgactccaccggcaagatcctggagcagcggagcctgaacaccatccagcagtttgattaccagaagaagctggacaacagggagaaggagagggtggcagcaaggcaggcctggtctgtggtgggcacaatcaaggatctgaagcagggctatctgagccaggtcatccacgagatcgtggacctgatgatccactaccaggccgtggtggtgctggagaacctgaatttcggctttaagagcaagaggaccggcatcgccgagaaggccgtgtaccagcagttcgagaagatgctgatcgataagctgaattgcctggtgctgaaggactatccagcagagaaagtgggaggcgtgctgaacccataccagctgacagaccagttcacctcctttgccaagatgggcacccagtctggcttcctgttttacgtgcctgccccatatacatctaagatcgatcccctgaccggcttcgtggaccccttcgtgtggaaaaccatcaagaatcacgagagccgcaagcacttcctggagggcttcgactttctgcactacgacgtgaaaaccggcgacttcatcctgcactttaagatgaacagaaatctgtccttccagaggggcctgcccggctttatgcctgcatgggatatcgtgttcgagaagaacgagacacagtttgacgccaagggcacccctttcatcgccggcaagagaatcgtgccagtgatcgagaatcacagattcaccggcagataccgggacctgtatcctgccaacgagctgatcgccctgctggaggagaagggcatcgtgttcagggatggctccaacatcctgccaaagctgctggagaatgacgattctcacgccatcgacaccatggtggccctgatccgcagcgtgctgcagatgcggaactccaatgccgccacaggcgaggactatatcaacagccccgtgcgcgatctgaatggcgtgtgcttcgactcccggtttcagaacccagagtggcccatggacgccgatgccaatggcgcctaccacatcgccctgaagggccagctgctgctgaatcacctgaaggagagcaaggatctgaagctgcagaacggcatctccaatcaggactggctggcctacatccaggagctgcgcaacaaaaggccggcggccacgaaaaaggccggccaggcaaaaaagaaaaagggatcctacccatacgatgttccagattacgcttatccctacgacgtgcctgattatgcatacccatatgatgtccccgactatgcctaagaattctgcagatatccagcacagtggcggccgctcgagtctagagggcccgtttaaacccgctgatcagcctcgactgtgccttctagttgccagccatctgttgtttgcccctcccccgtgccttccttgaccctggaaggtgccactcccactgtcctttcctaataaaatgaggaaattgcatcgcattgtctgagtaggtgtcattctattctggggggtggggtggggcaggacagcaagggggaggattgggaagacaatagcaggcatgctggggatgcggtgggctctatggcttctgaggcggaaagaaccagctggggctctagggggtatccccacgcgccctgtagcggcgcattaagcgcggcgggtgtggtggttacgcgcagcgtgaccgctacacttgccagcgccctagcgcccgctcctttcgctttcttcccttcctttctcgccacgttcgccggctttccccgtcaagctctaaatcgggggctccctttagggttccgatttagtgctttacggcacctcgaccccaaaaaacttgattagggtgatggttcacgtagtgggccatcgccctgatagacggtttttcgccctttgacgttggagtccacgttctttaatagtggactcttgttccaaactggaacaacactcaaccctatctcggtctattcttttgatttataagggattttgccgatttcggcctattggttaaaaaatgagctgatttaacaaaaatttaacgcgaattaattctgtggaatgtgtgtcagttagggtgtggaaagtccccaggctccccagcaggcagaagtatgcaaagcatgcatctcaattagtcagcaaccaggtgtggaaagtccccaggctccccagcaggcagaagtatgcaaagcatgcatctcaattagtcagcaaccatagtcccgcccctaactccgcccatcccgcccctaactccgcccagttccgcccattctccgccccatggctgactaattttttttatttatgcagaggccgaggccgcctctgcctctgagctattccagaagtagtgaggaggcttttttggaggcctaggcttttgcaaaaagctcccgggagcttgtatatccattttcggatctgatcaagagacaggatgaggatcgtttcgcatgattgaacaagatggattgcacgcaggttctccggccgcttgggtggagaggctattcggctatgactgggcacaacagacaatcggctgctctgatgccgccgtgttccggctgtcagcgcaggggcgcccggttctttttgtcaagaccgacctgtccggtgccctgaatgaactgcaggacgaggcagcgcggctatcgtggctggccacgacgggcgttccttgcgcagctgtgctcgacgttgtcactgaagcgggaagggactggctgctattgggcgaagtgccggggcaggatctcctgtcatctcaccttgctcctgccgagaaagtatccatcatggctgatgcaatgcggcggctgcatacgcttgatccggctacctgcccattcgaccaccaagcgaaacatcgcatcgagcgagcacgtactcggatggaagccggtcttgtcgatcaggatgatctggacgaagagcatcaggggctcgcgccagccgaactgttcgccaggctcaaggcgcgcatgcccgacggcgaggatctcgtcgtgacccatggcgatgcctgcttgccgaatatcatggtggaaaatggccgcttttctggattcatcgactgtggccggctgggtgtggcggaccgctatcaggacatagcgttggctacccgtgatattgctgaagagcttggcggcgaatgggctgaccgcttcctcgtgctttacggtatcgccgctcccgattcgcagcgcatcgccttctatcgccttcttgacgagttcttctgagcgggactctggggttcgaaatgaccgaccaagcgacgcccaacctgccatcacgagatttcgattccaccgccgccttctatgaaaggttgggcttcggaatcgttttccgggacgccggctggatgatcctccagcgcggggatctcatgctggagttcttcgcccaccccaacttgtttattgcagcttataatggttacaaataaagcaatagcatcacaaatttcacaaataaagcatttttttcactgcattctagttgtggtttgtccaaactcatcaatgtatcttatcatgtctgtataccgtcgacctctagctagagcttggcgtaatcatggtcatagctgtttcctgtgtgaaattgttatccgctcacaattccacacaacatacgagccggaagcataaagtgtaaagcctggggtgcctaatgagtgagctaactcacattaattgcgttgcgctcactgcccgctttccagtcgggaaacctgtcgtgccagctgcattaatgaatcggccaacgcgcggggagaggcggtttgcgtattgggcgctcttccgcttcctcgctcactgactcgctgcgctcggtcgttcggctgcggcgagcggtatcagctcactcaaaggcggtaatacggttatccacagaatcaggggataacgcaggaaagaacatgtgagcaaaaggccagcaaaaggccaggaaccgtaaaaaggccgcgttgctggcgtttttccataggctccgcccccctgacgagcatcacaaaaatcgacgctcaagtcagaggtggcgaaacccgacaggactataaagataccaggcgtttccccctggaagctccctcgtgcgctctcctgttccgaccctgccgcttaccggatacctgtccgcctttctcccttcgggaagcgtggcgctttctcatagctcacgctgtaggtatctcagttcggtgtaggtcgttcgctccaagctgggctgtgtgcacgaaccccccgttcagcccgaccgctgcgccttatccggtaactatcgtcttgagtccaacccggtaagacacgacttatcgccactggcagcagccactggtaacaggattagcagagcgaggtatgtaggcggtgctacagagttcttgaagtggtggcctaactacggctacactagaagaacagtatttggtatctgcgctctgctgaagccagttaccttcggaaaaagagttggtagctcttgatccggcaaacaaaccaccgctggtagcggtttttttgtttgcaagcagcagattacgcgcagaaaaaaaggatctcaagaagatcctttgatcttttctacggggtctgacgctcagtggaacgaaaactcacgttaagggattttggtcatgagattatcaaaaaggatcttcacctagatccttttaaattaaaaatgaagttttaaatcaatctaaagtatatatgagtaaacttggtctgacagttaccaatgcttaatcagtgaggcacctatctcagcgatctgtctatttcgttcatccatagttgcctgactccccgtcgtgtagataactacgatacgggagggcttaccatctggccccagtgctgcaatgataccgcgagacccacgctcaccggctccagatttatcagcaataaaccagccagccggaagggccgagcgcagaagtggtcctgcaactttatccgcctccatccagtctattaattgttgccgggaagctagagtaagtagttcgccagttaatagtttgcgcaacgttgttgccattgctacaggcatcgtggtgtcacgctcgtcgtttggtatggcttcattcagctccggttcccaacgatcaaggcgagttacatgatcccccatgttgtgcaaaaaagcggttagctccttcggtcctccgatcgttgtcagaagtaagttggccgcagtgttatcactcatggttatggcagcactgcataattctcttactgtcatgccatccgtaagatgcttttctgtgactggtgagtactcaaccaagtcattctgagaatagtgtatgcggcgaccgagttgctcttgcccggcgtcaatacgggataataccgcgccacatagcagaactttaaaagtgctcatcattggaaaacgttcttcggggcgaaaactctcaaggatcttaccgctgttgagatccagttcgatgtaacccactcgtgcacccaactgatcttcagcatcttttactttcaccagcgtttctgggtgagcaaaaacaggaaggcaaaatgccgcaaaaaagggaataagggcgacacggaaatgttgaatactcatactcttcctttttcaatattattgaagcatttatcagggttattgtctcatgagcggatacatatttgaatgtatttagaaaaataaacaaataggggttccgcgcacatttccccgaaaagtgccacctgacgtc

SEQ ID NO: 125 - DNA, 9227 bp, synthetic construct
  source 1..9227: mol_type = other DNA
gacggatcgggagatctcccgatcccctatggtgcactctcagtacaatctgctctgatgccgcatagttaagccagtatctgctccctgcttgtgtgttggaggtcgctgagtagtgcgcgagcaaaatttaagctacaacaaggcaaggcttgaccgacaattgcatgaagaatctgcttagggttaggcgttttgcgctgcttcgcgatgtacgggccagatatacgcgttgacattgattattgactagttattaatagtaatcaattacggggtcattagttcatagcccatatatggagttccgcgttacataacttacggtaaatggcccgcctggctgaccgcccaacgacccccgcccattgacgtcaataatgacgtatgttcccatagtaacgccaatagggactttccattgacgtcaatgggtggagtatttacggtaaactgcccacttggcagtacatcaagtgtatcatatgccaagtacgccccctattgacgtcaatgacggtaaatggcccgcctggcattatgcccagtacatgaccttatgggactttcctacttggcagtacatctacgtattagtcatcgctattaccatggtgatgcggttttggcagtacatcaatgggcgtggatagcggtttgactcacggggatttccaagtctccaccccattgacgtcaatgggagtttgttttggcaccaaaatcaacgggactttccaaaatgtcgtaacaactccgccccattgacgcaaatgggcggtaggcgtgtacggtgggaggtctatataagcagagctctctggctaactagagaacccactgcttactggcttatcgaaattaatacgactcactatagggagacccaagctggctagcgtttaaacttaagcttggtaccgccaccatgagcaagctggagaagtttacaaactgctactccctgtctaagaccctgaggttcaaggccatccctgtgggcaagacccaggagaacatcgacaataagcggctgctggtggaggacgagaagagagccgaggattataagggcgtgaagaagctgctggatcgctactatctgtcttttatcaacgacgtgctgcacagcatcaagctgaagaatctgaacaattacatcagcctgttccggaagaaaaccagaaccgagaaggagaataaggagctggagaacctggagatcaatctgcggaaggagatcgccaaggccttcaagggcaacgagggctacaagtccctgtttaagaaggatatcatcgagacaatcctgccagagttcctggacgataaggacgagatcgccctggtgaacagcttcaatggctttaccacagccttcaccggcttctttgataacagagagaatatgttttccgaggaggccaagagcacatccatcgccttcaggtgtatcaacgagaatctgacccgctacatctctaatatggacatcttcgagaaggtggacgccatctttgataagcacgaggtgcaggagatcaaggagaagatcctgaacagcgactatgatgtggaggatttctttgagggcgagttctttaactttgtgctgacacaggagggcatcgacgtgtataacgccatcatcggcggcttcgtgaccgagagcggcgagaagatcaagggcctgaacgagtacatcaacctgtataatcagaaaaccaagcagaagctgcctaagtttaagccactgtataagcaggtgctgagcgatcgggagtctctgagcttctacggcgagggctatacatccgatgaggaggtgctggaggtgtttagaaacaccctgaacaagaacagcgagatcttcagctccatcaagaagctggagaagctgttcaagaattttgacgagtactctagcgccggcatctttgtgaagaacggccccgccatcagcacaatctccaaggatatcttcggcgagtggaacgtgatccgggacaagtggaatgccgagtatgacgatatccacctgaagaagaaggccgtggtgaccgagaagtacgaggacgatcggagaaagtccttcaagaagatcggctccttttctctggagcagctgcaggagtacgccgacgccgatctgtctgtggtggagaagctgaaggagatcatcatccagaaggtggatgagatctacaaggtgtatggctcctctgagaagctgttcgacgccgattttgtgctggagaagagcctgaagaagaacgacgccgtggtggccatcatgaaggacctgctggattctgtgaagagcttcgagaattacatcaaggccttctttggcgagggcaaggagacaaacagggacgagtccttctatggcgattttgtgctggcctacgacatcctgctgaaggtggaccacatctacgatgccatccgcaattatgtgacccagaagccctactctaaggataagttcaagctgtattttcagaaccctcagttcatgggcggctgggacaaggataaggagacagactatcgggccaccatcctgagatacggctccaagtactatctggccatcatggataagaagtacgccaagtgcctgcagaagatcgacaaggacgatgtgaacggcaattacgagaagatcaactataagctgctgcccggccctaataagatgctgccaaaggtgttcttttctaagaagtggatggcctactataaccccagcgaggacatccagaagatctacaagaatggcacattcaagaagggcgatatgtttaacctgaatgactgtcacaagctgatcgacttctttaaggatagcatctcccggtatccaaagtggtccaatgcctacgatttcaacttttctgagacagagaagtataaggacatcgccggcttttacagagaggtggaggagcagggctataaggtgagcttcgagtctgccagcaagaaggaggtggataagctggtggaggagggcaagctgtatatgttccagatctataacaaggacttttccgataagtctcacggcacacccaatctgcacaccatgtacttcaagctgctgtttgacgagaacaatcacggacagatcaggctgagcggaggagcagagctgttcatgaggcgcgcctccctgaagaaggaggagctggtggtgcacccagccaactcccctatcgccaacaagaatccagataatcccaagaaaaccacaaccctgtcctacgacgtgtataaggataagaggttttctgaggaccagtacgagctgcacatcccaatcgccatcaataagtgccccaagaacatcttcaagatcaatacagaggtgcgcgtgctgctgaagcacgacgataacccctatgtgatcggcatcgataggggcgagcgcaatctgctgtatatcgtggtggtggacggcaagggcaacatcgtggagcagtattccctgaacgagatcatcaacaacttcaacggcatcaggatcaagacagattaccactctctgctggacaagaaggagaaggagaggttcgaggcccgccagaactggacctccatcgagaatatcaaggagctgaaggccggctatatctctcaggtggtgcacaagatctgcgagctggtggagaagtacgatgccgtgatcgccctggaggacctgaactctggctttaagaatagccgcgtgaaggtggagaagcaggtgtatcagaagttcgagaagatgctgatcgataagctgaactacatggtggacaagaagtctaatccttgtgcaacaggcggcgccctgaagggctatcagatcaccaataagttcgagagctttaagtccatgtctacccagaacggcttcatcttttacatccctgcctggctgacatccaagatcgatccatctaccggctttgtgaacctgctgaaaaccaagtataccagcatcgccgattccaagaagttcatcagctcctttgacaggatcatgtacgtgcccgaggaggatctgttcgagtttgccctggactataagaacttctctcgcacagacgccgattacatcaagaagtggaagctgtactcctacggcaaccggatcagaatcttccggaatcctaagaagaacaacgtgttcgactgggaggaggtgtgcctgaccagcgcctataaggagctgttcaacaagtacggcatcaattatcagcagggcgatatcagagccctgctgtgcgagcagtccgacaaggccttctactctagctttatggccctgatgagcctgatgctgcagatgcggaacagcatcacaggccgcaccgacgtggattttctgatcagccctgtgaagaactccgacggcatcttctacgatagccggaactatgaggcccaggagaatgccatcctgccaaagaacgccgacgccaatggcgcctataacatcgccagaaaggtgctgtgggccatcggccagttcaagaaggccgaggacgagaagctggataaggtgaagatcgccatctctaacaaggagtggctggagtacgcccagaccagcgtgaagcacaaaaggccggcggccacgaaaaaggccggccaggcaaaaaagaaaaagggatcctacccatacgatgttccagattacgcttatccctacgacgtgcctgattatgcatacccatatgatgtccccgactatgcctaagaattctgcagatatccagcacagtggcggccgctcgagtctagagggcccgtttaaacccgctgatcagcctcgactgtgccttctagttgccagccatctgttgtttgcccctcccccgtgccttccttgaccctggaaggtgccactcccactgtcctttcctaataaaatgaggaaattgcatcgcattgtctgagtaggtgtcattctattctggggggtggggtggggcaggacagcaagggggaggattgggaagacaatagcaggcatgctggggatgcggtgggctctatggcttctgaggcggaaagaaccagctggggctctagggggtatccccacgcgccctgtagcggcgcattaagcgcggcgggtgtggtggttacgcgcagcgtgaccgctacacttgccagcgccctagcgcccgctcctttcgctttcttcccttcctttctcgccacgttcgccggctttccccgtcaagctctaaatcgggggctccctttagggttccgatttagtgctttacggcacctcgaccccaaaaaacttgattagggtgatggttcacgtagtgggccatcgccctgatagacggtttttcgccctttgacgttggagtccacgttctttaatagtggactcttgttccaaactggaacaacactcaaccctatctcggtctattcttttgatttataagggattttgccgatttcggcctattggttaaaaaatgagctgatttaacaaaaatttaacgcgaattaattctgtggaatgtgtgtcagttagggtgtggaaagtccccaggctccccagcaggcagaagtatgcaaagcatgcatctcaattagtcagcaaccaggtgtggaaagtccccaggctccccagcaggcagaagtatgcaaagcatgcatctcaattagtcagcaaccatagtcccgcccctaactccgcccatcccgcccctaactccgcccagttccgcccattctccgccccatggctgactaattttttttatttatgcagaggccgaggccgcctctgcctctgagctattccagaagtagtgaggaggcttttttggaggcctaggcttttgcaaaaagctcccgggagcttgtatatccattttcggatctgatcaagagacaggatgaggatcgtttcgcatgattgaacaagatggattgcacgcaggttctccggccgcttgggtggagaggctattcggctatgactgggcacaacagacaatcggctgctctgatgccgccgtgttccggctgtcagcgcaggggcgcccggttctttttgtcaagaccgacctgtccggtgccctgaatgaactgcaggacgaggcagcgcggctatcgtggctggccacgacgggcgttccttgcgcagctgtgctcgacgttgtcactgaagcgggaagggactggctgctattgggcgaagtgccggggcaggatctcctgtcatctcaccttgctcctgccgagaaagtatccatcatggctgatgcaatgcggcggctgcatacgcttgatccggctacctgcccattcgaccaccaagcgaaacatcgcatcgagcgagcacgtactcggatggaagccggtcttgtcgatcaggatgatctggacgaagagcatcaggggctcgcgccagccgaactgttcgccaggctcaaggcgcgcatgcccgacggcgaggatctcgtcgtgacccatggcgatgcctgcttgccgaatatcatggtggaaaatggccgcttttctggattcatcgactgtggccggctgggtgtggcggaccgctatcaggacatagcgttggctacccgtgatattgctgaagagcttggcggcgaatgggctgaccgcttcctcgtgctttacggtatcgccgctcccgattcgcagcgcatcgccttctatcgccttcttgacgagttcttctgagcgggactctggggttcgaaatgaccgaccaagcgacgcccaacctgccatcacgagatttcgattccaccgccgccttctatgaaaggttgggcttcggaatcgttttccgggacgccggctggatgatcctccagcgcggggatctcatgctggagttcttcgcccaccccaacttgtttattgcagcttataatggttacaaataaagcaatagcatcacaaatttcacaaataaagcatttttttcactgcattctagttgtggtttgtccaaactcatcaatgtatcttatcatgtctgtataccgtcgacctctagctagagcttggcgtaatcatggtcatagctgtttcctgtgtgaaattgttatccgctcacaattccacacaacatacgagccggaagcataaagtgtaaagcctggggtgcctaatgagtgagctaactcacattaattgcgttgcgctcactgcccgctttccagtcgggaaacctgtcgtgccagctgcattaatgaatcggccaacgcgcggggagaggcggtttgcgtattgggcgctcttccgcttcctcgctcactgactcgctgcgctcggtcgttcggctgcggcgagcggtatcagctcactcaaaggcggtaatacggttatccacagaatcaggggataacgcaggaaagaacatgtgagcaaaaggccagcaaaaggccaggaaccgtaaaaaggccgcgttgctggcgtttttccataggctccgcccccctgacgagcatcacaaaaatcgacgctcaagtcagaggtggcgaaacccgacaggactataaagataccaggcgtttccccctggaagctccctcgtgcgctctcctgttccgaccctgccgcttaccggatacctgtccgcctttctcccttcgggaagcgtggcgctttctcatagctcacgctgtaggtatctcagttcggtgtaggtcgttcgctccaagctgggctgtgtgcacgaaccccccgttcagcccgaccgctgcgccttatccggtaactatcgtcttgagtccaacccggtaagacacgacttatcgccactggcagcagccactggtaacaggattagcagagcgaggtatgtaggcggtgctacagagttcttgaagtggtggcctaactacggctacactagaagaacagtatttggtatctgcgctctgctgaagccagttaccttcggaaaaagagttggtagctcttgatccggcaaacaaaccaccgctggtagcggtttttttgtttgcaagcagcagattacgcgcagaaaaaaaggatctcaagaagatcctttgatcttttctacggggtctgacgctcagtggaacgaaaactcacgttaagggattttggtcatgagattatcaaaaaggatcttcacctagatccttttaaattaaaaatgaagttttaaatcaatctaaagtatatatgagtaaacttggtctgacagttaccaatgcttaatcagtgaggcacctatctcagcgatctgtctatttcgttcatccatagttgcctgactccccgtcgtgtagataactacgatacgggagggcttaccatctggccccagtgctgcaatgataccgcgagacccacgctcaccggctccagatttatcagcaataaaccagccagccggaagggccgagcgcagaagtggtcctgcaactttatccgcctccatccagtctattaattgttgccgggaagctagagtaagtagttcgccagttaatagtttgcgcaacgttgttgccattgctacaggcatcgtggtgtcacgctcgtcgtttggtatggcttcattcagctccggttcccaacgatcaaggcgagttacatgatcccccatgttgtgcaaaaaagcggttagctccttcggtcctccgatcgttgtcagaagtaagttggccgcagtgttatcactcatggttatggcagcactgcataattctcttactgtcatgccatccgtaagatgcttttctgtgactggtgagtactcaaccaagtcattctgagaatagtgtatgcggcgaccgagttgctcttgcccggcgtcaatacgggataataccgcgccacatagcagaactttaaaagtgctcatcattggaaaacgttcttcggggcgaaaactctcaaggatcttaccgctgttgagatccagttcgatgtaacccactcgtgcacccaactgatcttcagcatcttttactttcaccagcgtttctgggtgagcaaaaacaggaaggcaaaatgccgcaaaaaagggaataagggcgacacggaaatgttgaatactcatactcttcctttttcaatattattgaagcatttatcagggttattgtctcatgagcggatacatatttgaatgtatttagaaaaataaacaaataggggttccgcgcacatttccccgaaaagtgccacctgacgtc